European Patent Specification EP 3 458 477 B1, published July 9, 2025. Title: ANTI-FACTOR IX PADUA ANTIBODIES. Applicant: BAXALTA INCORPORATED BAXALTA GMBH. The sequence listing filed with the application follows.

SEQUENCE LISTING (28 sequences)

SEQ ID NO: 1 - protein, 461 aa, Homo sapiens
MQRVNMIMAESPGLITICLLGYLLSAECTVFLDHENANKILNRPKRYNSGKLEEFVQGNLERECMEEKCSFEEAREVFENTERTTEFWKQYVDGDQCESNPCLNGGSCKDDINSYECWCPFGFEGKNCELDVTCNIKNGRCEQFCKNSADNKVVCSCTEGYRLAENQKSCEPAVPFPCGRVSVSQTSKLTRAETVFPDVDYVNSTEAETILDNITQSTQSFNDFTRVVGGEDAKPGQFPWQVVLNGKVDAFCGGSIVNEKWIVTAAHCVETGVKITVVAGEHNIEETEHTEQKRNVIRIIPHHNYNAAINKYNHDIALLELDEPLVLNSYVTPICIADKEYTNIFLKFGSGYVSGWGRVFHKGRSALVLQYLRVPLVDRATCLLSTKFTIYNNMFCAGFHEGGRDSCQGDSGGPHVTEVEGTSFLTGIISWGEECAMKGKYGIYTKVSRYVNWIKEKTKLT

SEQ ID NO: 2 - protein, 461 aa, Homo sapiens
MQRVNMIMAESPGLITICLLGYLLSAECTVFLDHENANKILNRPKRYNSGKLEEFVQGNLERECMEEKCSFEEAREVFENTERTTEFWKQYVDGDQCESNPCLNGGSCKDDINSYECWCPFGFEGKNCELDVTCNIKNGRCEQFCKNSADNKVVCSCTEGYRLAENQKSCEPAVPFPCGRVSVSQTSKLTRAETVFPDVDYVNSTEAETILDNITQSTQSFNDFTRVVGGEDAKPGQFPWQVVLNGKVDAFCGGSIVNEKWIVTAAHCVETGVKITVVAGEHNIEETEHTEQKRNVIRIIPHHNYNAAINKYNHDIALLELDEPLVLNSYVTPICIADKEYTNIFLKFGSGYVSGWGRVFHKGRSALVLQYLRVPLVDRATCLRSTKFTIYNNMFCAGFHEGGRDSCQGDSGGPHVTEVEGTSFLTGIISWGEECAMKGKYGIYTKVSRYVNWIKEKTKLT

SEQ ID NO: 3 - protein, 12 aa, Homo sapiens
DRATCLLSTKFT

SEQ ID NO: 4 - protein, 26 aa, Homo sapiens
LVDRATCLLSTKFTIYNNMFCAGFHE

SEQ ID NO: 5 - protein, 25 aa, Homo sapiens
LVDRATCLLSTKFTIYNNMFCAGFH

SEQ ID NO: 6 - protein, 6 aa, Homo sapiens
SSYAIS

SEQ ID NO: 7 - protein, 17 aa, Homo sapiens
GIVPAFGTANYAQKFQG

SEQ ID NO: 8 - protein, 9 aa, Homo sapiens
SWGVISFAY

SEQ ID NO: 9 - protein, 11 aa, Homo sapiens
RASQDISSYLN

SEQ ID NO: 10 - protein, 7 aa, Homo sapiens
AASNLQS

SEQ ID NO: 11 - protein, 10 aa, Homo sapiens
MQYDSLPFTF

SEQ ID NO: 12 - protein, 8 aa, Homo sapiens
DYKDDDDK

SEQ ID NO: 13 - protein, 6 aa, Homo sapiens
HHHHHH

SEQ ID NO: 14 - protein, 12 aa, Homo sapiens
DRATCLRSTKFT

SEQ ID NO: 15 - protein, 25 aa, Homo sapiens
LVDRATCLRSTKFTIYNNMFCAGFH

SEQ ID NO: 16 - protein, 622 aa, Homo sapiens
  ref <308>: GenBank / AAH51332.1
  ref <309>: 2006-07-15
  ref <313>: (1)..(622)
MAHVRGLQLPGCLALAALCSLVHSQHVFLAPQQARSLLQRVRRANTFLEEVRKGNLERECVEETCSYEEAFEALESSTATDVFWAKYTACETARTPRDKLAACLEGNCAEGLGTNYRGHVNITRSGIECQLWRSRYPHKPEINSTTHPGADLQENFCRNPDSSTTGPWCYTTDPTVRRQECSIPVCGQDQVTVAMTPRSEGSSVNLSPPLEQCVPDRGQQYQGRLAVTTHGLPCLAWASAQAKALSKHQDFNSAVQLVENFCRNPDGDEEGAWCYVAGKPGDFGYCDLNYCEEAVEEETGDGLDEDSDRAIEGRTATSEYQTFFNPRTFGSGEADCGLRPLFEKKSLEDKTERELLESYIDGRIVEGSDAEIGMSPWQVMLFRKSPQELLCGASLISDRWVLTAAHCLLYPPWDKNFTENDLLVRIGKHSRTRYERNIEKISMLEKIYIHPRYNWRENLDRDIALMKLKKPVAFSDYIHPVCLPDRETAASLLQAGYKGRVTGWGNLKETWTANVGKGQPSVLQVVNLPIVERPVCKDSTRIRITDNMFCAGYKPDEGKRGDACEGDSGGPFVMKSPFNNRWYQMGIVSWGEGCDRDGKYGFYTHVFRLKKWIQKVIDQFGE

SEQ ID NO: 17 - protein, 467 aa, Homo sapiens
  ref <308>: PRF / 1205236A
  ref <309>: 1996-10-18
  ref <313>: (1)..(467)
LLGESLFIRREQANNILARVTRANSFLEEMKKGHLERECMEETCSYEEAREVFEDSDKTNEFWNKYKDGDQCETSPCQNQGKCKDGLGEYTCTCLEGFEGKNCELFTRKLCSLDNGDCDQFCHEEQNSVVCSCARGYTLADNGKACIPTGPYPCGKQTLERRKRSVAQATSSSGEAPDSITWKPYDAADLDPTENPFDLLDFNQTQPERGDNNLTRIVGGQECKDGECPWQALLINEENEGFCGGTILSEFYILTAAHCLYQAKRFEGDRNTEQEEGGEAVHEVEVVIKHNRFTKETYDFDIAVLRLKTPITFRMNVAPACLPERDWAESTLMTQKTGIVSGFGRTHEKGRQSTRLKMLEVPYVDRNSCKLSSSFIITQNMFCAGYDTKQEDACQGDSGGPHVTRFKDTYFVTGIVSWGEGCARKGKYGIYTKVTAFLKWIDRSMKTRGLPKAKSHAPEVITSSPLK

SEQ ID NO: 18-23 - skipped (6 entries)

SEQ ID NO: 24 - protein, 118 aa, Homo sapiens
QVQLVQSGAEVKKPGSSVKVSCKASGGTFSSYAISWVRQAPGQGLEWMGGIVPAFGTANYAQKFQGRVTITADESTSTAYMELSSLRSEDTAVYYCARSWGVISFAYWGQGTLVTVSS

SEQ ID NO: 25 - protein, 109 aa, Homo sapiens
DIQMTQSPSSLSASVGDRVTITCRASQDISSYLNWYQQKPGKAPKLLIYAASNLQSGVPSRFSGSGSGTDFTLTISSLQPEDFATYYCMQYDSLPFTFGQGTKVEIKRT

SEQ ID NO: 26 - protein, 220 aa, Homo sapiens
QVQLVQSGAEVKKPGSSVKVSCKASGGTFSSYAISWVRQAPGQGLEWMGGIVPAFGTANYAQKFQGRVTITADESTSTAYMELSSLRSEDTAVYYCARSWGVISFAYWGQGTLVTVSSASTKGPSVFPLAPSSKSTSGGTAALGCLVKDYFPEPVTVSWNSGALTSGVHTFPAVLQSSGLYSLSSVVTVPSSSLGTQTYICNVNHKPSNTKVDKKVEPKS

SEQ ID NO: 27 - protein, 214 aa, Homo sapiens
DIQMTQSPSSLSASVGDRVTITCRASQDISSYLNWYQQKPGKAPKLLIYAASNLQSGVPSRFSGSGSGTDFTLTISSLQPEDFATYYCMQYDSLPFTFGQGTKVEIKRTVAAPSVFIFPPSDEQLKSGTASVVCLLNNFYPREAKVQWKVDNALQSGNSQESVTEQDSKDSTYSLSSTLTLSKADYEKHKVYACEVTHQGLSSPVTKSFNRGEA

SEQ ID NO: 28 - protein, 290 aa, Homo sapiens
QVQLVQSGAEVKKPGSSVKVSCKASGGTFSSYAISWVRQAPGQGLEWMGGIVPAFGTANYAQKFQGRVTITADESTSTAYMELSSLRSEDTAVYYCARSWGVISFAYWGQGTLVTVSSASTKGPSVFPLAPSSKSTSGGTAALGCLVKDYFPEPVTVSWNSGALTSGVHTFPAVLQSSGLYSLSSVVTVPSSSLGTQTYICNVNHKPSNTKVDKKVEPKSEFPKPSTPPGSSGELEELLKHLKELLKGPRKGELEELLKHLKELLKGGSGGAPDYKDDDDKDAPHHHHHH